European Patent Specification EP 3 511 424 B1, published October 18, 2023. Title: Compositions and Methods for Improving Nanopore Sequencing. Applicant: University of Washington through its Center for Commercialization. Application EP13825899.1. The sequence listing filed with the application follows.

SEQUENCE LISTING (3 sequences)

SEQ ID NO: 1 - DNA, 93 bp, Artificial Sequence
  Synthetic
  misc_feature (14)..(14): Wheren N at position 14 = X representing an abasic residue
aaaaaaaccttccnagaccaatcaagcaactaattaagtaacgaatgaaggaacaaataaagaaaaccaagcattctcatgcaggtcgtagcc

SEQ ID NO: 2 - DNA, 43 bp, Artificial Sequence
  Synthetic
  misc_feature (37)..(43): Wherein N at positions 37-43 = X representing an abasic residue
ttggttttctttatttgttccttcattcgttacttannnnnnn

SEQ ID NO: 3 - DNA, 55 bp, Artificial Sequence
  Synthetic
gcgtacgcctacggttttccgtaggcgtacgcggctacgacctgcatgagaatgc